European Patent Specification EP 3 362 557 B1, published October 25, 2023. Title: Mutant  beta-glucosidase variants with increased thermostability. Applicant: Technische Universität München. The sequence listing filed with the application follows.

SEQUENCE LISTING (52 sequences)

SEQ ID NO: 1 - protein, 447 aa, Artificial Sequence
  Synthetic polypeptide
  VARIANT (40)..(40): Xaa is selected from Glu, Pro, Thr, Met, Ala, Ser and Gly
  VARIANT (111)..(111): Xaa is selected from Val, Lys, Arg and His
  VARIANT (293)..(293): Xaa is selected from Val, Ile, Leu, Met, Pro, Thr and Ala
  VARIANT (423)..(423): Xaa is selected from Thr, Glu, Asp, Asn, Gln, Met and Pro
  VARIANT (441)..(441): Xaa is selected from Leu, Arg, Lys and His
MAKFPRDFVWGTATSSYQIEGAVNEDGRTPSIWDTFSKTXGKTYKGHTGDVACDHYHRYKEDVEILKEIGVKAYRFSIAWPRIFPEEGKYNPKGMDFYKKLIDELQKRDIXPAATIYHWDLPQWAYDKGGGWLNRESIKWYVEYATKLFEELGDAIPLWITHNEPWCSSILSYGIGEHAPGHKNYREALIAAHHILLSHGEAVKAFREMNIKGSKIGITLNLTPAYPASEKEEDKLAAQYADGFANRWFLDPIFKGNYPEDMMELYSKIIGEFDFIKEGDLETISVPIDFLGXNYYTRSIVKYDEDSMLKAENVPGPGKRTEMGWEISPESLYDLLKRLDREYTKLPMYITENGAAFKDEVTEDGRVHDDERIEYIKEHLKAAAKFIGEGGNLKGYFVWSLMDNFEWAHGYSKRFGIVYVDYXTQKRILKDSALWYKEVIXDDGIED

SEQ ID NO: 2 - protein, 447 aa, Artificial Sequence
  Synthetic Polypeptide
  Variant (111)..(111): Xaa is selected from Val, Lys, Arg and His
  Variant (293)..(293): Xaa is selected from Val, Ile, Leu, Met, Pro, Thr and Ala
  Variant (423)..(423): Xaa is selected from Thr, Glu, Asp, Asn, Gln, Met and Pro
  Variant (441)..(441): Xaa is selected from Leu, Arg, Lys and His
MAKFPRDFVWGTATSSYQIEGAVNEDGRTPSIWDTFSKTPGKTYKGHTGDVACDHYHRYKEDVEILKEIGVKAYRFSIAWPRIFPEEGKYNPKGMDFYKKLIDELQKRDIXPAATIYHWDLPQWAYDKGGGWLNRESIKWYVEYATKLFEELGDAIPLWITHNEPWCSSILSYGIGEHAPGHKNYREALIAAHHILLSHGEAVKAFREMNIKGSKIGITLNLTPAYPASEKEEDKLAAQYADGFANRWFLDPIFKGNYPEDMMELYSKIIGEFDFIKEGDLETISVPIDFLGXNYYTRSIVKYDEDSMLKAENVPGPGKRTEMGWEISPESLYDLLKRLDREYTKLPMYITENGAAFKDEVTEDGRVHDDERIEYIKEHLKAAAKFIGEGGNLKGYFVWSLMDNFEWAHGYSKRFGIVYVDYXTQKRILKDSALWYKEVIXDDGIED

SEQ ID NO: 3 - protein, 447 aa, Artificial Sequence
  Synthetic Polypeptide
  Variant (40)..(40): Xaa is selected from Glu, Pro, Thr, Met, Ala, Ser and Gly
  Variant (293)..(293): Xaa is selected from Val, Ile, Leu, Met, Pro, Thr and Ala
  Variant (423)..(423): Xaa is selected from Thr, Glu, Asp, Asn, Gln, Met and Pro
  Variant (441)..(441): Xaa is selected from Leu, Arg, Lys and His
MAKFPRDFVWGTATSSYQIEGAVNEDGRTPSIWDTFSKTXGKTYKGHTGDVACDHYHRYKEDVEILKEIGVKAYRFSIAWPRIFPEEGKYNPKGMDFYKKLIDELQKRDIKPAATIYHWDLPQWAYDKGGGWLNRESIKWYVEYATKLFEELGDAIPLWITHNEPWCSSILSYGIGEHAPGHKNYREALIAAHHILLSHGEAVKAFREMNIKGSKIGITLNLTPAYPASEKEEDKLAAQYADGFANRWFLDPIFKGNYPEDMMELYSKIIGEFDFIKEGDLETISVPIDFLGXNYYTRSIVKYDEDSMLKAENVPGPGKRTEMGWEISPESLYDLLKRLDREYTKLPMYITENGAAFKDEVTEDGRVHDDERIEYIKEHLKAAAKFIGEGGNLKGYFVWSLMDNFEWAHGYSKRFGIVYVDYXTQKRILKDSALWYKEVIXDDGIED

SEQ ID NO: 4 - protein, 447 aa, Artificial Sequence
  Synthetic Polypeptide
  Variant (40)..(40): Xaa is selected from Glu, Pro, Thr, Met, Ala, Ser and Gly
  Variant (111)..(111): Xaa is selected from Val, Lys, Arg and His
  Variant (423)..(423): Xaa is selected from Thr, Glu, Asp, Asn, Gln, Met and Pro
  Variant (441)..(441): Xaa is selected from Leu, Arg, Lys and His
MAKFPRDFVWGTATSSYQIEGAVNEDGRTPSIWDTFSKTXGKTYKGHTGDVACDHYHRYKEDVEILKEIGVKAYRFSIAWPRIFPEEGKYNPKGMDFYKKLIDELQKRDIXPAATIYHWDLPQWAYDKGGGWLNRESIKWYVEYATKLFEELGDAIPLWITHNEPWCSSILSYGIGEHAPGHKNYREALIAAHHILLSHGEAVKAFREMNIKGSKIGITLNLTPAYPASEKEEDKLAAQYADGFANRWFLDPIFKGNYPEDMMELYSKIIGEFDFIKEGDLETISVPIDFLGINYYTRSIVKYDEDSMLKAENVPGPGKRTEMGWEISPESLYDLLKRLDREYTKLPMYITENGAAFKDEVTEDGRVHDDERIEYIKEHLKAAAKFIGEGGNLKGYFVWSLMDNFEWAHGYSKRFGIVYVDYXTQKRILKDSALWYKEVIXDDGIED

SEQ ID NO: 5 - protein, 447 aa, Artificial Sequence
  Synthetic Polypeptide
  Variant (40)..(40): Xaa is selected from Glu, Pro, Thr, Met, Ala, Ser and Gly
  Variant (111)..(111): Xaa is selected from Val, Lys, Arg and His
  Variant (293)..(293): Xaa is selected from Val, Ile, Leu, Met, Pro, Thr and Ala
  Variant (441)..(441): Xaa is selected from Leu, Arg, Lys and His
MAKFPRDFVWGTATSSYQIEGAVNEDGRTPSIWDTFSKTXGKTYKGHTGDVACDHYHRYKEDVEILKEIGVKAYRFSIAWPRIFPEEGKYNPKGMDFYKKLIDELQKRDIXPAATIYHWDLPQWAYDKGGGWLNRESIKWYVEYATKLFEELGDAIPLWITHNEPWCSSILSYGIGEHAPGHKNYREALIAAHHILLSHGEAVKAFREMNIKGSKIGITLNLTPAYPASEKEEDKLAAQYADGFANRWFLDPIFKGNYPEDMMELYSKIIGEFDFIKEGDLETISVPIDFLGXNYYTRSIVKYDEDSMLKAENVPGPGKRTEMGWEISPESLYDLLKRLDREYTKLPMYITENGAAFKDEVTEDGRVHDDERIEYIKEHLKAAAKFIGEGGNLKGYFVWSLMDNFEWAHGYSKRFGIVYVDYETQKRILKDSALWYKEVIXDDGIED

SEQ ID NO: 6 - protein, 447 aa, Artificial Sequence
  Synthetic Polypeptide
  Variant (40)..(40): Xaa is selected from Glu, Pro, Thr, Met, Ala, Ser and Gly
  Variant (111)..(111): X is selected from V, K, R and H
  Variant (293)..(293): Xaa is selected from Val, Ile, Leu, Met, Pro, Thr and Ala
  Variant (423)..(423): Xaa is selected from Thr, Glu, Asp, Asn, Gln, Met and Pro
MAKFPRDFVWGTATSSYQIEGAVNEDGRTPSIWDTFSKTXGKTYKGHTGDVACDHYHRYKEDVEILKEIGVKAYRFSIAWPRIFPEEGKYNPKGMDFYKKLIDELQKRDIXPAATIYHWDLPQWAYDKGGGWLNRESIKWYVEYATKLFEELGDAIPLWITHNEPWCSSILSYGIGEHAPGHKNYREALIAAHHILLSHGEAVKAFREMNIKGSKIGITLNLTPAYPASEKEEDKLAAQYADGFANRWFLDPIFKGNYPEDMMELYSKIIGEFDFIKEGDLETISVPIDFLGXNYYTRSIVKYDEDSMLKAENVPGPGKRTEMGWEISPESLYDLLKRLDREYTKLPMYITENGAAFKDEVTEDGRVHDDERIEYIKEHLKAAAKFIGEGGNLKGYFVWSLMDNFEWAHGYSKRFGIVYVDYXTQKRILKDSALWYKEVIRDDGIED

SEQ ID NO: 7 - protein, 447 aa, Artificial Sequence
  Synthetic Polypeptide
MAKFPRDFVWGTATSSYQIEGAVNEDGRTPSIWDTFSKTPGKTYKGHTGDVACDHYHRYKEDVEILKEIGVKAYRFSIAWPRIFPEEGKYNPKGMDFYKKLIDELQKRDIVPAATIYHWDLPQWAYDKGGGWLNRESIKWYVEYATKLFEELGDAIPLWITHNEPWCSSILSYGIGEHAPGHKNYREALIAAHHILLSHGEAVKAFREMNIKGSKIGITLNLTPAYPASEKEEDKLAAQYADGFANRWFLDPIFKGNYPEDMMELYSKIIGEFDFIKEGDLETISVPIDFLGVNYYTRSIVKYDEDSMLKAENVPGPGKRTEMGWEISPESLYDLLKRLDREYTKLPMYITENGAAFKDEVTEDGRVHDDERIEYIKEHLKAAAKFIGEGGNLKGYFVWSLMDNFEWAHGYSKRFGIVYVDYTTQKRILKDSALWYKEVILDDGIED

SEQ ID NO: 8 - protein, 447 aa, Artificial Sequence
  Synthetic Polypeptide
MAKFPRDFVWGTATSSYQIEGAVNEDGRTPSIWDTFSKTEGKTYKGHTGDVACDHYHRYKEDVEILKEIGVKAYRFSIAWPRIFPEEGKYNPKGMDFYKKLIDELQKRDIKPAATIYHWDLPQWAYDKGGGWLNRESIKWYVEYATKLFEELGDAIPLWITHNEPWCSSILSYGIGEHAPGHKNYREALIAAHHILLSHGEAVKAFREMNIKGSKIGITLNLTPAYPASEKEEDKLAAQYADGFANRWFLDPIFKGNYPEDMMELYSKIIGEFDFIKEGDLETISVPIDFLGVNYYTRSIVKYDEDSMLKAENVPGPGKRTEMGWEISPESLYDLLKRLDREYTKLPMYITENGAAFKDEVTEDGRVHDDERIEYIKEHLKAAAKFIGEGGNLKGYFVWSLMDNFEWAHGYSKRFGIVYVDYTTQKRILKDSALWYKEVILDDGIED

SEQ ID NO: 9 - protein, 447 aa, Artificial Sequence
  Synthetic Polypeptide
MAKFPRDFVWGTATSSYQIEGAVNEDGRTPSIWDTFSKTEGKTYKGHTGDVACDHYHRYKEDVEILKEIGVKAYRFSIAWPRIFPEEGKYNPKGMDFYKKLIDELQKRDIVPAATIYHWDLPQWAYDKGGGWLNRESIKWYVEYATKLFEELGDAIPLWITHNEPWCSSILSYGIGEHAPGHKNYREALIAAHHILLSHGEAVKAFREMNIKGSKIGITLNLTPAYPASEKEEDKLAAQYADGFANRWFLDPIFKGNYPEDMMELYSKIIGEFDFIKEGDLETISVPIDFLGINYYTRSIVKYDEDSMLKAENVPGPGKRTEMGWEISPESLYDLLKRLDREYTKLPMYITENGAAFKDEVTEDGRVHDDERIEYIKEHLKAAAKFIGEGGNLKGYFVWSLMDNFEWAHGYSKRFGIVYVDYTTQKRILKDSALWYKEVILDDGIED

SEQ ID NO: 10 - protein, 447 aa, Artificial Sequence
  Synthetic Polypeptide
MAKFPRDFVWGTATSSYQIEGAVNEDGRTPSIWDTFSKTEGKTYKGHTGDVACDHYHRYKEDVEILKEIGVKAYRFSIAWPRIFPEEGKYNPKGMDFYKKLIDELQKRDIVPAATIYHWDLPQWAYDKGGGWLNRESIKWYVEYATKLFEELGDAIPLWITHNEPWCSSILSYGIGEHAPGHKNYREALIAAHHILLSHGEAVKAFREMNIKGSKIGITLNLTPAYPASEKEEDKLAAQYADGFANRWFLDPIFKGNYPEDMMELYSKIIGEFDFIKEGDLETISVPIDFLGVNYYTRSIVKYDEDSMLKAENVPGPGKRTEMGWEISPESLYDLLKRLDREYTKLPMYITENGAAFKDEVTEDGRVHDDERIEYIKEHLKAAAKFIGEGGNLKGYFVWSLMDNFEWAHGYSKRFGIVYVDYETQKRILKDSALWYKEVILDDGIED

SEQ ID NO: 11 - protein, 447 aa, Artificial Sequence
  Synthetic Polypeptide
MAKFPRDFVWGTATSSYQIEGAVNEDGRTPSIWDTFSKTEGKTYKGHTGDVACDHYHRYKEDVEILKEIGVKAYRFSIAWPRIFPEEGKYNPKGMDFYKKLIDELQKRDIVPAATIYHWDLPQWAYDKGGGWLNRESIKWYVEYATKLFEELGDAIPLWITHNEPWCSSILSYGIGEHAPGHKNYREALIAAHHILLSHGEAVKAFREMNIKGSKIGITLNLTPAYPASEKEEDKLAAQYADGFANRWFLDPIFKGNYPEDMMELYSKIIGEFDFIKEGDLETISVPIDFLGVNYYTRSIVKYDEDSMLKAENVPGPGKRTEMGWEISPESLYDLLKRLDREYTKLPMYITENGAAFKDEVTEDGRVHDDERIEYIKEHLKAAAKFIGEGGNLKGYFVWSLMDNFEWAHGYSKRFGIVYVDYTTQKRILKDSALWYKEVIRDDGIED

SEQ ID NO: 12 - protein, 447 aa, Artificial Sequence
  Synthetic Polypeptide
MAKFPRDFVWGTATSSYQIEGAVNEDGRTPSIWDTFSKTPGKTYKGHTGDVACDHYHRYKEDVEILKEIGVKAYRFSIAWPRIFPEEGKYNPKGMDFYKKLIDELQKRDIKPAATIYHWDLPQWAYDKGGGWLNRESIKWYVEYATKLFEELGDAIPLWITHNEPWCSSILSYGIGEHAPGHKNYREALIAAHHILLSHGEAVKAFREMNIKGSKIGITLNLTPAYPASEKEEDKLAAQYADGFANRWFLDPIFKGNYPEDMMELYSKIIGEFDFIKEGDLETISVPIDFLGVNYYTRSIVKYDEDSMLKAENVPGPGKRTEMGWEISPESLYDLLKRLDREYTKLPMYITENGAAFKDEVTEDGRVHDDERIEYIKEHLKAAAKFIGEGGNLKGYFVWSLMDNFEWAHGYSKRFGIVYVDYTTQKRILKDSALWYKEVILDDGIED

SEQ ID NO: 13 - protein, 447 aa, Artificial Sequence
  Synthetic Polypeptide
MAKFPRDFVWGTATSSYQIEGAVNEDGRTPSIWDTFSKTPGKTYKGHTGDVACDHYHRYKEDVEILKEIGVKAYRFSIAWPRIFPEEGKYNPKGMDFYKKLIDELQKRDIVPAATIYHWDLPQWAYDKGGGWLNRESIKWYVEYATKLFEELGDAIPLWITHNEPWCSSILSYGIGEHAPGHKNYREALIAAHHILLSHGEAVKAFREMNIKGSKIGITLNLTPAYPASEKEEDKLAAQYADGFANRWFLDPIFKGNYPEDMMELYSKIIGEFDFIKEGDLETISVPIDFLGINYYTRSIVKYDEDSMLKAENVPGPGKRTEMGWEISPESLYDLLKRLDREYTKLPMYITENGAAFKDEVTEDGRVHDDERIEYIKEHLKAAAKFIGEGGNLKGYFVWSLMDNFEWAHGYSKRFGIVYVDYTTQKRILKDSALWYKEVILDDGIED

SEQ ID NO: 14 - protein, 447 aa, Artificial Sequence
  Synthetic Polypeptide
MAKFPRDFVWGTATSSYQIEGAVNEDGRTPSIWDTFSKTPGKTYKGHTGDVACDHYHRYKEDVEILKEIGVKAYRFSIAWPRIFPEEGKYNPKGMDFYKKLIDELQKRDIVPAATIYHWDLPQWAYDKGGGWLNRESIKWYVEYATKLFEELGDAIPLWITHNEPWCSSILSYGIGEHAPGHKNYREALIAAHHILLSHGEAVKAFREMNIKGSKIGITLNLTPAYPASEKEEDKLAAQYADGFANRWFLDPIFKGNYPEDMMELYSKIIGEFDFIKEGDLETISVPIDFLGVNYYTRSIVKYDEDSMLKAENVPGPGKRTEMGWEISPESLYDLLKRLDREYTKLPMYITENGAAFKDEVTEDGRVHDDERIEYIKEHLKAAAKFIGEGGNLKGYFVWSLMDNFEWAHGYSKRFGIVYVDYETQKRILKDSALWYKEVILDDGIED

SEQ ID NO: 15 - protein, 447 aa, Artificial Sequence
  Synthetic Polypeptide
MAKFPRDFVWGTATSSYQIEGAVNEDGRTPSIWDTFSKTPGKTYKGHTGDVACDHYHRYKEDVEILKEIGVKAYRFSIAWPRIFPEEGKYNPKGMDFYKKLIDELQKRDIVPAATIYHWDLPQWAYDKGGGWLNRESIKWYVEYATKLFEELGDAIPLWITHNEPWCSSILSYGIGEHAPGHKNYREALIAAHHILLSHGEAVKAFREMNIKGSKIGITLNLTPAYPASEKEEDKLAAQYADGFANRWFLDPIFKGNYPEDMMELYSKIIGEFDFIKEGDLETISVPIDFLGVNYYTRSIVKYDEDSMLKAENVPGPGKRTEMGWEISPESLYDLLKRLDREYTKLPMYITENGAAFKDEVTEDGRVHDDERIEYIKEHLKAAAKFIGEGGNLKGYFVWSLMDNFEWAHGYSKRFGIVYVDYTTQKRILKDSALWYKEVIRDDGIED

SEQ ID NO: 16 - protein, 447 aa, Artificial Sequence
  Synthetic Polypeptide
MAKFPRDFVWGTATSSYQIEGAVNEDGRTPSIWDTFSKTEGKTYKGHTGDVACDHYHRYKEDVEILKEIGVKAYRFSIAWPRIFPEEGKYNPKGMDFYKKLIDELQKRDIKPAATIYHWDLPQWAYDKGGGWLNRESIKWYVEYATKLFEELGDAIPLWITHNEPWCSSILSYGIGEHAPGHKNYREALIAAHHILLSHGEAVKAFREMNIKGSKIGITLNLTPAYPASEKEEDKLAAQYADGFANRWFLDPIFKGNYPEDMMELYSKIIGEFDFIKEGDLETISVPIDFLGINYYTRSIVKYDEDSMLKAENVPGPGKRTEMGWEISPESLYDLLKRLDREYTKLPMYITENGAAFKDEVTEDGRVHDDERIEYIKEHLKAAAKFIGEGGNLKGYFVWSLMDNFEWAHGYSKRFGIVYVDYTTQKRILKDSALWYKEVILDDGIED

SEQ ID NO: 17 - protein, 447 aa, Artificial Sequence
  Synthetic Polypeptide
MAKFPRDFVWGTATSSYQIEGAVNEDGRTPSIWDTFSKTEGKTYKGHTGDVACDHYHRYKEDVEILKEIGVKAYRFSIAWPRIFPEEGKYNPKGMDFYKKLIDELQKRDIKPAATIYHWDLPQWAYDKGGGWLNRESIKWYVEYATKLFEELGDAIPLWITHNEPWCSSILSYGIGEHAPGHKNYREALIAAHHILLSHGEAVKAFREMNIKGSKIGITLNLTPAYPASEKEEDKLAAQYADGFANRWFLDPIFKGNYPEDMMELYSKIIGEFDFIKEGDLETISVPIDFLGVNYYTRSIVKYDEDSMLKAENVPGPGKRTEMGWEISPESLYDLLKRLDREYTKLPMYITENGAAFKDEVTEDGRVHDDERIEYIKEHLKAAAKFIGEGGNLKGYFVWSLMDNFEWAHGYSKRFGIVYVDYETQKRILKDSALWYKEVILDDGIED

SEQ ID NO: 18 - protein, 447 aa, Artificial Sequence
  Synthetic Polypeptide
MAKFPRDFVWGTATSSYQIEGAVNEDGRTPSIWDTFSKTEGKTYKGHTGDVACDHYHRYKEDVEILKEIGVKAYRFSIAWPRIFPEEGKYNPKGMDFYKKLIDELQKRDIKPAATIYHWDLPQWAYDKGGGWLNRESIKWYVEYATKLFEELGDAIPLWITHNEPWCSSILSYGIGEHAPGHKNYREALIAAHHILLSHGEAVKAFREMNIKGSKIGITLNLTPAYPASEKEEDKLAAQYADGFANRWFLDPIFKGNYPEDMMELYSKIIGEFDFIKEGDLETISVPIDFLGVNYYTRSIVKYDEDSMLKAENVPGPGKRTEMGWEISPESLYDLLKRLDREYTKLPMYITENGAAFKDEVTEDGRVHDDERIEYIKEHLKAAAKFIGEGGNLKGYFVWSLMDNFEWAHGYSKRFGIVYVDYTTQKRILKDSALWYKEVIRDDGIED

SEQ ID NO: 19 - protein, 447 aa, Artificial Sequence
  Synthetic Polypeptide
MAKFPRDFVWGTATSSYQIEGAVNEDGRTPSIWDTFSKTEGKTYKGHTGDVACDHYHRYKEDVEILKEIGVKAYRFSIAWPRIFPEEGKYNPKGMDFYKKLIDELQKRDIVPAATIYHWDLPQWAYDKGGGWLNRESIKWYVEYATKLFEELGDAIPLWITHNEPWCSSILSYGIGEHAPGHKNYREALIAAHHILLSHGEAVKAFREMNIKGSKIGITLNLTPAYPASEKEEDKLAAQYADGFANRWFLDPIFKGNYPEDMMELYSKIIGEFDFIKEGDLETISVPIDFLGINYYTRSIVKYDEDSMLKAENVPGPGKRTEMGWEISPESLYDLLKRLDREYTKLPMYITENGAAFKDEVTEDGRVHDDERIEYIKEHLKAAAKFIGEGGNLKGYFVWSLMDNFEWAHGYSKRFGIVYVDYETQKRILKDSALWYKEVILDDGIED

SEQ ID NO: 20 - protein, 447 aa, Artificial Sequence
  Synthetic Polypeptide
MAKFPRDFVWGTATSSYQIEGAVNEDGRTPSIWDTFSKTEGKTYKGHTGDVACDHYHRYKEDVEILKEIGVKAYRFSIAWPRIFPEEGKYNPKGMDFYKKLIDELQKRDIVPAATIYHWDLPQWAYDKGGGWLNRESIKWYVEYATKLFEELGDAIPLWITHNEPWCSSILSYGIGEHAPGHKNYREALIAAHHILLSHGEAVKAFREMNIKGSKIGITLNLTPAYPASEKEEDKLAAQYADGFANRWFLDPIFKGNYPEDMMELYSKIIGEFDFIKEGDLETISVPIDFLGINYYTRSIVKYDEDSMLKAENVPGPGKRTEMGWEISPESLYDLLKRLDREYTKLPMYITENGAAFKDEVTEDGRVHDDERIEYIKEHLKAAAKFIGEGGNLKGYFVWSLMDNFEWAHGYSKRFGIVYVDYTTQKRILKDSALWYKEVIRDDGIED

SEQ ID NO: 21 - protein, 447 aa, Artificial Sequence
  Synthetic Poylpeptide
MAKFPRDFVWGTATSSYQIEGAVNEDGRTPSIWDTFSKTEGKTYKGHTGDVACDHYHRYKEDVEILKEIGVKAYRFSIAWPRIFPEEGKYNPKGMDFYKKLIDELQKRDIVPAATIYHWDLPQWAYDKGGGWLNRESIKWYVEYATKLFEELGDAIPLWITHNEPWCSSILSYGIGEHAPGHKNYREALIAAHHILLSHGEAVKAFREMNIKGSKIGITLNLTPAYPASEKEEDKLAAQYADGFANRWFLDPIFKGNYPEDMMELYSKIIGEFDFIKEGDLETISVPIDFLGVNYYTRSIVKYDEDSMLKAENVPGPGKRTEMGWEISPESLYDLLKRLDREYTKLPMYITENGAAFKDEVTEDGRVHDDERIEYIKEHLKAAAKFIGEGGNLKGYFVWSLMDNFEWAHGYSKRFGIVYVDYETQKRILKDSALWYKEVIRDDGIED

SEQ ID NO: 22 - protein, 447 aa, Artificial Sequence
  Synthetic Polypeptide
MAKFPRDFVWGTATSSYQIEGAVNEDGRTPSIWDTFSKTPGKTYKGHTGDVACDHYHRYKEDVEILKEIGVKAYRFSIAWPRIFPEEGKYNPKGMDFYKKLIDELQKRDIKPAATIYHWDLPQWAYDKGGGWLNRESIKWYVEYATKLFEELGDAIPLWITHNEPWCSSILSYGIGEHAPGHKNYREALIAAHHILLSHGEAVKAFREMNIKGSKIGITLNLTPAYPASEKEEDKLAAQYADGFANRWFLDPIFKGNYPEDMMELYSKIIGEFDFIKEGDLETISVPIDFLGINYYTRSIVKYDEDSMLKAENVPGPGKRTEMGWEISPESLYDLLKRLDREYTKLPMYITENGAAFKDEVTEDGRVHDDERIEYIKEHLKAAAKFIGEGGNLKGYFVWSLMDNFEWAHGYSKRFGIVYVDYTTQKRILKDSALWYKEVILDDGIED

SEQ ID NO: 23 - protein, 447 aa, Artificial Sequence
  Synthetic Polypeptide
MAKFPRDFVWGTATSSYQIEGAVNEDGRTPSIWDTFSKTPGKTYKGHTGDVACDHYHRYKEDVEILKEIGVKAYRFSIAWPRIFPEEGKYNPKGMDFYKKLIDELQKRDIKPAATIYHWDLPQWAYDKGGGWLNRESIKWYVEYATKLFEELGDAIPLWITHNEPWCSSILSYGIGEHAPGHKNYREALIAAHHILLSHGEAVKAFREMNIKGSKIGITLNLTPAYPASEKEEDKLAAQYADGFANRWFLDPIFKGNYPEDMMELYSKIIGEFDFIKEGDLETISVPIDFLGVNYYTRSIVKYDEDSMLKAENVPGPGKRTEMGWEISPESLYDLLKRLDREYTKLPMYITENGAAFKDEVTEDGRVHDDERIEYIKEHLKAAAKFIGEGGNLKGYFVWSLMDNFEWAHGYSKRFGIVYVDYETQKRILKDSALWYKEVILDDGIED

SEQ ID NO: 24 - protein, 447 aa, Artificial Sequence
  Synthetic Polypeptide
MAKFPRDFVWGTATSSYQIEGAVNEDGRTPSIWDTFSKTPGKTYKGHTGDVACDHYHRYKEDVEILKEIGVKAYRFSIAWPRIFPEEGKYNPKGMDFYKKLIDELQKRDIKPAATIYHWDLPQWAYDKGGGWLNRESIKWYVEYATKLFEELGDAIPLWITHNEPWCSSILSYGIGEHAPGHKNYREALIAAHHILLSHGEAVKAFREMNIKGSKIGITLNLTPAYPASEKEEDKLAAQYADGFANRWFLDPIFKGNYPEDMMELYSKIIGEFDFIKEGDLETISVPIDFLGVNYYTRSIVKYDEDSMLKAENVPGPGKRTEMGWEISPESLYDLLKRLDREYTKLPMYITENGAAFKDEVTEDGRVHDDERIEYIKEHLKAAAKFIGEGGNLKGYFVWSLMDNFEWAHGYSKRFGIVYVDYTTQKRILKDSALWYKEVIRDDGIED

SEQ ID NO: 25 - protein, 447 aa, Artificial Sequence
  Synthetic Polypeptide
MAKFPRDFVWGTATSSYQIEGAVNEDGRTPSIWDTFSKTPGKTYKGHTGDVACDHYHRYKEDVEILKEIGVKAYRFSIAWPRIFPEEGKYNPKGMDFYKKLIDELQKRDIVPAATIYHWDLPQWAYDKGGGWLNRESIKWYVEYATKLFEELGDAIPLWITHNEPWCSSILSYGIGEHAPGHKNYREALIAAHHILLSHGEAVKAFREMNIKGSKIGITLNLTPAYPASEKEEDKLAAQYADGFANRWFLDPIFKGNYPEDMMELYSKIIGEFDFIKEGDLETISVPIDFLGINYYTRSIVKYDEDSMLKAENVPGPGKRTEMGWEISPESLYDLLKRLDREYTKLPMYITENGAAFKDEVTEDGRVHDDERIEYIKEHLKAAAKFIGEGGNLKGYFVWSLMDNFEWAHGYSKRFGIVYVDYETQKRILKDSALWYKEVILDDGIED

SEQ ID NO: 26 - protein, 447 aa, Artificial Sequence
  Synthetic Polypeptide
MAKFPRDFVWGTATSSYQIEGAVNEDGRTPSIWDTFSKTPGKTYKGHTGDVACDHYHRYKEDVEILKEIGVKAYRFSIAWPRIFPEEGKYNPKGMDFYKKLIDELQKRDIVPAATIYHWDLPQWAYDKGGGWLNRESIKWYVEYATKLFEELGDAIPLWITHNEPWCSSILSYGIGEHAPGHKNYREALIAAHHILLSHGEAVKAFREMNIKGSKIGITLNLTPAYPASEKEEDKLAAQYADGFANRWFLDPIFKGNYPEDMMELYSKIIGEFDFIKEGDLETISVPIDFLGINYYTRSIVKYDEDSMLKAENVPGPGKRTEMGWEISPESLYDLLKRLDREYTKLPMYITENGAAFKDEVTEDGRVHDDERIEYIKEHLKAAAKFIGEGGNLKGYFVWSLMDNFEWAHGYSKRFGIVYVDYTTQKRILKDSALWYKEVIRDDGIED

SEQ ID NO: 27 - protein, 447 aa, Artificial Sequence
  Synthetic Polypeptide
MAKFPRDFVWGTATSSYQIEGAVNEDGRTPSIWDTFSKTPGKTYKGHTGDVACDHYHRYKEDVEILKEIGVKAYRFSIAWPRIFPEEGKYNPKGMDFYKKLIDELQKRDIVPAATIYHWDLPQWAYDKGGGWLNRESIKWYVEYATKLFEELGDAIPLWITHNEPWCSSILSYGIGEHAPGHKNYREALIAAHHILLSHGEAVKAFREMNIKGSKIGITLNLTPAYPASEKEEDKLAAQYADGFANRWFLDPIFKGNYPEDMMELYSKIIGEFDFIKEGDLETISVPIDFLGVNYYTRSIVKYDEDSMLKAENVPGPGKRTEMGWEISPESLYDLLKRLDREYTKLPMYITENGAAFKDEVTEDGRVHDDERIEYIKEHLKAAAKFIGEGGNLKGYFVWSLMDNFEWAHGYSKRFGIVYVDYETQKRILKDSALWYKEVIRDDGIED

SEQ ID NO: 28 - protein, 447 aa, Artificial Sequence
  Synthetic Polypeptide
MAKFPRDFVWGTATSSYQIEGAVNEDGRTPSIWDTFSKTEGKTYKGHTGDVACDHYHRYKEDVEILKEIGVKAYRFSIAWPRIFPEEGKYNPKGMDFYKKLIDELQKRDIKPAATIYHWDLPQWAYDKGGGWLNRESIKWYVEYATKLFEELGDAIPLWITHNEPWCSSILSYGIGEHAPGHKNYREALIAAHHILLSHGEAVKAFREMNIKGSKIGITLNLTPAYPASEKEEDKLAAQYADGFANRWFLDPIFKGNYPEDMMELYSKIIGEFDFIKEGDLETISVPIDFLGINYYTRSIVKYDEDSMLKAENVPGPGKRTEMGWEISPESLYDLLKRLDREYTKLPMYITENGAAFKDEVTEDGRVHDDERIEYIKEHLKAAAKFIGEGGNLKGYFVWSLMDNFEWAHGYSKRFGIVYVDYETQKRILKDSALWYKEVILDDGIED

SEQ ID NO: 29 - protein, 447 aa, Artificial Sequence
  Synthetic Poylpeptide
MAKFPRDFVWGTATSSYQIEGAVNEDGRTPSIWDTFSKTEGKTYKGHTGDVACDHYHRYKEDVEILKEIGVKAYRFSIAWPRIFPEEGKYNPKGMDFYKKLIDELQKRDIKPAATIYHWDLPQWAYDKGGGWLNRESIKWYVEYATKLFEELGDAIPLWITHNEPWCSSILSYGIGEHAPGHKNYREALIAAHHILLSHGEAVKAFREMNIKGSKIGITLNLTPAYPASEKEEDKLAAQYADGFANRWFLDPIFKGNYPEDMMELYSKIIGEFDFIKEGDLETISVPIDFLGINYYTRSIVKYDEDSMLKAENVPGPGKRTEMGWEISPESLYDLLKRLDREYTKLPMYITENGAAFKDEVTEDGRVHDDERIEYIKEHLKAAAKFIGEGGNLKGYFVWSLMDNFEWAHGYSKRFGIVYVDYTTQKRILKDSALWYKEVIRDDGIED

SEQ ID NO: 30 - protein, 447 aa, Artificial Sequence
  Synthetic Polypeptide
MAKFPRDFVWGTATSSYQIEGAVNEDGRTPSIWDTFSKTEGKTYKGHTGDVACDHYHRYKEDVEILKEIGVKAYRFSIAWPRIFPEEGKYNPKGMDFYKKLIDELQKRDIKPAATIYHWDLPQWAYDKGGGWLNRESIKWYVEYATKLFEELGDAIPLWITHNEPWCSSILSYGIGEHAPGHKNYREALIAAHHILLSHGEAVKAFREMNIKGSKIGITLNLTPAYPASEKEEDKLAAQYADGFANRWFLDPIFKGNYPEDMMELYSKIIGEFDFIKEGDLETISVPIDFLGVNYYTRSIVKYDEDSMLKAENVPGPGKRTEMGWEISPESLYDLLKRLDREYTKLPMYITENGAAFKDEVTEDGRVHDDERIEYIKEHLKAAAKFIGEGGNLKGYFVWSLMDNFEWAHGYSKRFGIVYVDYETQKRILKDSALWYKEVIRDDGIED

SEQ ID NO: 31 - protein, 447 aa, Artificial Sequence
  Synthetic Polypeptide
MAKFPRDFVWGTATSSYQIEGAVNEDGRTPSIWDTFSKTEGKTYKGHTGDVACDHYHRYKEDVEILKEIGVKAYRFSIAWPRIFPEEGKYNPKGMDFYKKLIDELQKRDIVPAATIYHWDLPQWAYDKGGGWLNRESIKWYVEYATKLFEELGDAIPLWITHNEPWCSSILSYGIGEHAPGHKNYREALIAAHHILLSHGEAVKAFREMNIKGSKIGITLNLTPAYPASEKEEDKLAAQYADGFANRWFLDPIFKGNYPEDMMELYSKIIGEFDFIKEGDLETISVPIDFLGINYYTRSIVKYDEDSMLKAENVPGPGKRTEMGWEISPESLYDLLKRLDREYTKLPMYITENGAAFKDEVTEDGRVHDDERIEYIKEHLKAAAKFIGEGGNLKGYFVWSLMDNFEWAHGYSKRFGIVYVDYETQKRILKDSALWYKEVIRDDGIED

SEQ ID NO: 32 - protein, 447 aa, Artificial Sequence
  Synthetic Polypeptide
MAKFPRDFVWGTATSSYQIEGAVNEDGRTPSIWDTFSKTPGKTYKGHTGDVACDHYHRYKEDVEILKEIGVKAYRFSIAWPRIFPEEGKYNPKGMDFYKKLIDELQKRDIKPAATIYHWDLPQWAYDKGGGWLNRESIKWYVEYATKLFEELGDAIPLWITHNEPWCSSILSYGIGEHAPGHKNYREALIAAHHILLSHGEAVKAFREMNIKGSKIGITLNLTPAYPASEKEEDKLAAQYADGFANRWFLDPIFKGNYPEDMMELYSKIIGEFDFIKEGDLETISVPIDFLGINYYTRSIVKYDEDSMLKAENVPGPGKRTEMGWEISPESLYDLLKRLDREYTKLPMYITENGAAFKDEVTEDGRVHDDERIEYIKEHLKAAAKFIGEGGNLKGYFVWSLMDNFEWAHGYSKRFGIVYVDYETQKRILKDSALWYKEVILDDGIED

SEQ ID NO: 33 - protein, 447 aa, Artificial Sequence
  Synthetic Polypeptide
MAKFPRDFVWGTATSSYQIEGAVNEDGRTPSIWDTFSKTPGKTYKGHTGDVACDHYHRYKEDVEILKEIGVKAYRFSIAWPRIFPEEGKYNPKGMDFYKKLIDELQKRDIKPAATIYHWDLPQWAYDKGGGWLNRESIKWYVEYATKLFEELGDAIPLWITHNEPWCSSILSYGIGEHAPGHKNYREALIAAHHILLSHGEAVKAFREMNIKGSKIGITLNLTPAYPASEKEEDKLAAQYADGFANRWFLDPIFKGNYPEDMMELYSKIIGEFDFIKEGDLETISVPIDFLGINYYTRSIVKYDEDSMLKAENVPGPGKRTEMGWEISPESLYDLLKRLDREYTKLPMYITENGAAFKDEVTEDGRVHDDERIEYIKEHLKAAAKFIGEGGNLKGYFVWSLMDNFEWAHGYSKRFGIVYVDYTTQKRILKDSALWYKEVIRDDGIED

SEQ ID NO: 34 - protein, 447 aa, Artificial Sequence
  Synthetic Polypeptide
MAKFPRDFVWGTATSSYQIEGAVNEDGRTPSIWDTFSKTPGKTYKGHTGDVACDHYHRYKEDVEILKEIGVKAYRFSIAWPRIFPEEGKYNPKGMDFYKKLIDELQKRDIKPAATIYHWDLPQWAYDKGGGWLNRESIKWYVEYATKLFEELGDAIPLWITHNEPWCSSILSYGIGEHAPGHKNYREALIAAHHILLSHGEAVKAFREMNIKGSKIGITLNLTPAYPASEKEEDKLAAQYADGFANRWFLDPIFKGNYPEDMMELYSKIIGEFDFIKEGDLETISVPIDFLGVNYYTRSIVKYDEDSMLKAENVPGPGKRTEMGWEISPESLYDLLKRLDREYTKLPMYITENGAAFKDEVTEDGRVHDDERIEYIKEHLKAAAKFIGEGGNLKGYFVWSLMDNFEWAHGYSKRFGIVYVDYETQKRILKDSALWYKEVIRDDGIED

SEQ ID NO: 35 - protein, 447 aa, Artificial Sequence
  Synthetic Polypeptide
MAKFPRDFVWGTATSSYQIEGAVNEDGRTPSIWDTFSKTPGKTYKGHTGDVACDHYHRYKEDVEILKEIGVKAYRFSIAWPRIFPEEGKYNPKGMDFYKKLIDELQKRDIVPAATIYHWDLPQWAYDKGGGWLNRESIKWYVEYATKLFEELGDAIPLWITHNEPWCSSILSYGIGEHAPGHKNYREALIAAHHILLSHGEAVKAFREMNIKGSKIGITLNLTPAYPASEKEEDKLAAQYADGFANRWFLDPIFKGNYPEDMMELYSKIIGEFDFIKEGDLETISVPIDFLGINYYTRSIVKYDEDSMLKAENVPGPGKRTEMGWEISPESLYDLLKRLDREYTKLPMYITENGAAFKDEVTEDGRVHDDERIEYIKEHLKAAAKFIGEGGNLKGYFVWSLMDNFEWAHGYSKRFGIVYVDYETQKRILKDSALWYKEVIRDDGIED

SEQ ID NO: 36 - protein, 447 aa, Artificial Sequence
  Synthetic Polypeptide
MAKFPRDFVWGTATSSYQIEGAVNEDGRTPSIWDTFSKTEGKTYKGHTGDVACDHYHRYKEDVEILKEIGVKAYRFSIAWPRIFPEEGKYNPKGMDFYKKLIDELQKRDIKPAATIYHWDLPQWAYDKGGGWLNRESIKWYVEYATKLFEELGDAIPLWITHNEPWCSSILSYGIGEHAPGHKNYREALIAAHHILLSHGEAVKAFREMNIKGSKIGITLNLTPAYPASEKEEDKLAAQYADGFANRWFLDPIFKGNYPEDMMELYSKIIGEFDFIKEGDLETISVPIDFLGINYYTRSIVKYDEDSMLKAENVPGPGKRTEMGWEISPESLYDLLKRLDREYTKLPMYITENGAAFKDEVTEDGRVHDDERIEYIKEHLKAAAKFIGEGGNLKGYFVWSLMDNFEWAHGYSKRFGIVYVDYETQKRILKDSALWYKEVIRDDGIED

SEQ ID NO: 37 - protein, 447 aa, Artificial Sequence
  Synthetic Polypeptide
MAKFPRDFVWGTATSSYQIEGAVNEDGRTPSIWDTFSKTPGKTYKGHTGDVACDHYHRYKEDVEILKEIGVKAYRFSIAWPRIFPEEGKYNPKGMDFYKKLIDELQKRDIKPAATIYHWDLPQWAYDKGGGWLNRESIKWYVEYATKLFEELGDAIPLWITHNEPWCSSILSYGIGEHAPGHKNYREALIAAHHILLSHGEAVKAFREMNIKGSKIGITLNLTPAYPASEKEEDKLAAQYADGFANRWFLDPIFKGNYPEDMMELYSKIIGEFDFIKEGDLETISVPIDFLGINYYTRSIVKYDEDSMLKAENVPGPGKRTEMGWEISPESLYDLLKRLDREYTKLPMYITENGAAFKDEVTEDGRVHDDERIEYIKEHLKAAAKFIGEGGNLKGYFVWSLMDNFEWAHGYSKRFGIVYVDYETQKRILKDSALWYKEVIRDDGIED

SEQ ID NO: 38 - DNA, 1341 bp, Artificial Sequence
  Synthetic Polynucleotide
atggccaagtttcctcgcgactttgtatggggtacagccacatcgagttatcagattgaaggcgcggtgaatgaagatggtcgtacaccgtctatctgggacaccttttcgaaaaccgagggcaaaacctataaaggccatacgggtgatgttgcctgtgatcactatcaccgctataaggaagatgtggaaattctgaaagaaattggagtcaaagcctaccggtttagcattgcatggccacgtatctttcctgaggaaggcaaatacaacccgaaaggtatggatttctacaagaaactcattgacgaactgcaaaagcgcgatattgttcccgcagcgaccatttatcactgggatctgccacaatgggcctatgacaaaggcggtggctggctgaaccgtgagtccatcaaatggtatgtggagtacgcgaccaaattgtttgaagaactgggtgatgcgatcccgctgtggattacccataatgagccatggtgctcttctatcctcagttatggtatcggcgaacatgcacctggtcataagaactatcgcgaagcgcttattgctgcgcatcacatcctgctctcacatggcgaagcggtcaaagcgtttcgcgaaatgaacattaaggggagcaaaatcggcattacgcttaacttgactccggcgtatccagcaagtgagaaagaagaagataaactggctgcacagtatgcagatggctttgccaatcgctggttccttgacccgatcttcaagggtaactatccggaggacatgatggaattgtacagcaaaattattggggaattcgatttcattaaggaaggcgatctggagactatcagcgtcccgattgacttcttaggcgtcaattactacactcggagcattgttaaatacgatgaagattccatgctgaaagcagagaacgtaccgggaccgggtaaacgtaccgaaatggggtgggaaatctcgcccgagtcactgtacgacttactgaaacgcttagaccgtgagtatacgaaactgccgatgtatatcaccgaaaatggagctgcgtttaaagatgaagtaacggaagatggtcgtgttcacgacgatgaacgcatcgaatacatcaaagagcacctgaaagctgccgctaaatttatcggggaaggcggtaatctgaaaggatactttgtgtggtcattaatggacaacttcgaatgggcgcatggctactccaaacgtttcggcattgtgtatgtggactatacgacccagaaacgcattctgaaggatagcgccttgtggtacaaagaggtgattctggatgatgggattgaagat

SEQ ID NO: 39 - DNA, 1341 bp, Artificial Sequence
  Synthetic Polynucleotide
atggccaagtttcctcgcgactttgtatggggtacagccacatcgagttatcagattgaaggcgcggtgaatgaagatggtcgtacaccgtctatctgggacaccttttcgaaaaccccgggcaaaacctataaaggccatacgggtgatgttgcctgtgatcactatcaccgctataaggaagatgtggaaattctgaaagaaattggagtcaaagcctaccggtttagcattgcatggccacgtatctttcctgaggaaggcaaatacaacccgaaaggtatggatttctacaagaaactcattgacgaactgcaaaagcgcgatattgttcccgcagcgaccatttatcactgggatctgccacaatgggcctatgacaaaggcggtggctggctgaaccgtgagtccatcaaatggtatgtggagtacgcgaccaaattgtttgaagaactgggtgatgcgatcccgctgtggattacccataatgagccatggtgctcttctatcctcagttatggtatcggcgaacatgcacctggtcataagaactatcgcgaagcgcttattgctgcgcatcacatcctgctctcacatggcgaagcggtcaaagcgtttcgcgaaatgaacattaaggggagcaaaatcggcattacgcttaacttgactccggcgtatccagcaagtgagaaagaagaagataaactggctgcacagtatgcagatggctttgccaatcgctggttccttgacccgatcttcaagggtaactatccggaggacatgatggaattgtacagcaaaattattggggaattcgatttcattaaggaaggcgatctggagactatcagcgtcccgattgacttcttaggcgtcaattactacactcggagcattgttaaatacgatgaagattccatgctgaaagcagagaacgtaccgggaccgggtaaacgtaccgaaatggggtgggaaatctcgcccgagtcactgtacgacttactgaaacgcttagaccgtgagtatacgaaactgccgatgtatatcaccgaaaatggagctgcgtttaaagatgaagtaacggaagatggtcgtgttcacgacgatgaacgcatcgaatacatcaaagagcacctgaaagctgccgctaaatttatcggggaaggcggtaatctgaaaggatactttgtgtggtcattaatggacaacttcgaatgggcgcatggctactccaaacgtttcggcattgtgtatgtggactatacgacccagaaacgcattctgaaggatagcgccttgtggtacaaagaggtgattctggatgatgggattgaagat

SEQ ID NO: 40 - DNA, 1341 bp, Artificial Sequence
  Synthetic Polynucleotide
atggccaagtttcctcgcgactttgtatggggtacagccacatcgagttatcagattgaaggcgcggtgaatgaagatggtcgtacaccgtctatctgggacaccttttcgaaaaccgagggcaaaacctataaaggccatacgggtgatgttgcctgtgatcactatcaccgctataaggaagatgtggaaattctgaaagaaattggagtcaaagcctaccggtttagcattgcatggccacgtatctttcctgaggaaggcaaatacaacccgaaaggtatggatttctacaagaaactcattgacgaactgcaaaagcgcgatattaaacccgcagcgaccatttatcactgggatctgccacaatgggcctatgacaaaggcggtggctggctgaaccgtgagtccatcaaatggtatgtggagtacgcgaccaaattgtttgaagaactgggtgatgcgatcccgctgtggattacccataatgagccatggtgctcttctatcctcagttatggtatcggcgaacatgcacctggtcataagaactatcgcgaagcgcttattgctgcgcatcacatcctgctctcacatggcgaagcggtcaaagcgtttcgcgaaatgaacattaaggggagcaaaatcggcattacgcttaacttgactccggcgtatccagcaagtgagaaagaagaagataaactggctgcacagtatgcagatggctttgccaatcgctggttccttgacccgatcttcaagggtaactatccggaggacatgatggaattgtacagcaaaattattggggaattcgatttcattaaggaaggcgatctggagactatcagcgtcccgattgacttcttaggcgtcaattactacactcggagcattgttaaatacgatgaagattccatgctgaaagcagagaacgtaccgggaccgggtaaacgtaccgaaatggggtgggaaatctcgcccgagtcactgtacgacttactgaaacgcttagaccgtgagtatacgaaactgccgatgtatatcaccgaaaatggagctgcgtttaaagatgaagtaacggaagatggtcgtgttcacgacgatgaacgcatcgaatacatcaaagagcacctgaaagctgccgctaaatttatcggggaaggcggtaatctgaaaggatactttgtgtggtcattaatggacaacttcgaatgggcgcatggctactccaaacgtttcggcattgtgtatgtggactatacgacccagaaacgcattctgaaggatagcgccttgtggtacaaagaggtgattctggatgatgggattgaagat

SEQ ID NO: 41 - protein, 1341 aa, Artificial Sequence
  Synthetic Polynucleotide
ATGGCCAAGTTTCCTCGCGACTTTGTATGGGGTACAGCCACATCGAGTTATCAGATTGAAGGCGCGGTGAATGAAGATGGTCGTACACCGTCTATCTGGGACACCTTTTCGAAAACCGAGGGCAAAACCTATAAAGGCCATACGGGTGATGTTGCCTGTGATCACTATCACCGCTATAAGGAAGATGTGGAAATTCTGAAAGAAATTGGAGTCAAAGCCTACCGGTTTAGCATTGCATGGCCACGTATCTTTCCTGAGGAAGGCAAATACAACCCGAAAGGTATGGATTTCTACAAGAAACTCATTGACGAACTGCAAAAGCGCGATATTGTTCCCGCAGCGACCATTTATCACTGGGATCTGCCACAATGGGCCTATGACAAAGGCGGTGGCTGGCTGAACCGTGAGTCCATCAAATGGTATGTGGAGTACGCGACCAAATTGTTTGAAGAACTGGGTGATGCGATCCCGCTGTGGATTACCCATAATGAGCCATGGTGCTCTTCTATCCTCAGTTATGGTATCGGCGAACATGCACCTGGTCATAAGAACTATCGCGAAGCGCTTATTGCTGCGCATCACATCCTGCTCTCACATGGCGAAGCGGTCAAAGCGTTTCGCGAAATGAACATTAAGGGGAGCAAAATCGGCATTACGCTTAACTTGACTCCGGCGTATCCAGCAAGTGAGAAAGAAGAAGATAAACTGGCTGCACAGTATGCAGATGGCTTTGCCAATCGCTGGTTCCTTGACCCGATCTTCAAGGGTAACTATCCGGAGGACATGATGGAATTGTACAGCAAAATTATTGGGGAATTCGATTTCATTAAGGAAGGCGATCTGGAGACTATCAGCGTCCCGATTGACTTCTTAGGCATCAATTACTACACTCGGAGCATTGTTAAATACGATGAAGATTCCATGCTGAAAGCAGAGAACGTACCGGGACCGGGTAAACGTACCGAAATGGGGTGGGAAATCTCGCCCGAGTCACTGTACGACTTACTGAAACGCTTAGACCGTGAGTATACGAAACTGCCGATGTATATCACCGAAAATGGAGCTGCGTTTAAAGATGAAGTAACGGAAGATGGTCGTGTTCACGACGATGAACGCATCGAATACATCAAAGAGCACCTGAAAGCTGCCGCTAAATTTATCGGGGAAGGCGGTAATCTGAAAGGATACTTTGTGTGGTCATTAATGGACAACTTCGAATGGGCGCATGGCTACTCCAAACGTTTCGGCATTGTGTATGTGGACTATACGACCCAGAAACGCATTCTGAAGGATAGCGCCTTGTGGTACAAAGAGGTGATTCTGGATGATGGGATTGAAGAT

SEQ ID NO: 42 - DNA, 1341 bp, Artificial Sequence
  Synthetic Polynucleotide
atggccaagtttcctcgcgactttgtatggggtacagccacatcgagttatcagattgaaggcgcggtgaatgaagatggtcgtacaccgtctatctgggacaccttttcgaaaaccgagggcaaaacctataaaggccatacgggtgatgttgcctgtgatcactatcaccgctataaggaagatgtggaaattctgaaagaaattggagtcaaagcctaccggtttagcattgcatggccacgtatctttcctgaggaaggcaaatacaacccgaaaggtatggatttctacaagaaactcattgacgaactgcaaaagcgcgatattgttcccgcagcgaccatttatcactgggatctgccacaatgggcctatgacaaaggcggtggctggctgaaccgtgagtccatcaaatggtatgtggagtacgcgaccaaattgtttgaagaactgggtgatgcgatcccgctgtggattacccataatgagccatggtgctcttctatcctcagttatggtatcggcgaacatgcacctggtcataagaactatcgcgaagcgcttattgctgcgcatcacatcctgctctcacatggcgaagcggtcaaagcgtttcgcgaaatgaacattaaggggagcaaaatcggcattacgcttaacttgactccggcgtatccagcaagtgagaaagaagaagataaactggctgcacagtatgcagatggctttgccaatcgctggttccttgacccgatcttcaagggtaactatccggaggacatgatggaattgtacagcaaaattattggggaattcgatttcattaaggaaggcgatctggagactatcagcgtcccgattgacttcttaggcgtcaattactacactcggagcattgttaaatacgatgaagattccatgctgaaagcagagaacgtaccgggaccgggtaaacgtaccgaaatggggtgggaaatctcgcccgagtcactgtacgacttactgaaacgcttagaccgtgagtatacgaaactgccgatgtatatcaccgaaaatggagctgcgtttaaagatgaagtaacggaagatggtcgtgttcacgacgatgaacgcatcgaatacatcaaagagcacctgaaagctgccgctaaatttatcggggaaggcggtaatctgaaaggatactttgtgtggtcattaatggacaacttcgaatgggcgcatggctactccaaacgtttcggcattgtgtatgtggactatgagacccagaaacgcattctgaaggatagcgccttgtggtacaaagaggtgattctggatgatgggattgaagat

SEQ ID NO: 43 - DNA, 1341 bp, Artificial Sequence
  Synthetic Polynucleotide
atggccaagtttcctcgcgactttgtatggggtacagccacatcgagttatcagattgaaggcgcggtgaatgaagatggtcgtacaccgtctatctgggacaccttttcgaaaaccgagggcaaaacctataaaggccatacgggtgatgttgcctgtgatcactatcaccgctataaggaagatgtggaaattctgaaagaaattggagtcaaagcctaccggtttagcattgcatggccacgtatctttcctgaggaaggcaaatacaacccgaaaggtatggatttctacaagaaactcattgacgaactgcaaaagcgcgatattgttcccgcagcgaccatttatcactgggatctgccacaatgggcctatgacaaaggcggtggctggctgaaccgtgagtccatcaaatggtatgtggagtacgcgaccaaattgtttgaagaactgggtgatgcgatcccgctgtggattacccataatgagccatggtgctcttctatcctcagttatggtatcggcgaacatgcacctggtcataagaactatcgcgaagcgcttattgctgcgcatcacatcctgctctcacatggcgaagcggtcaaagcgtttcgcgaaatgaacattaaggggagcaaaatcggcattacgcttaacttgactccggcgtatccagcaagtgagaaagaagaagataaactggctgcacagtatgcagatggctttgccaatcgctggttccttgacccgatcttcaagggtaactatccggaggacatgatggaattgtacagcaaaattattggggaattcgatttcattaaggaaggcgatctggagactatcagcgtcccgattgacttcttaggcgtcaattactacactcggagcattgttaaatacgatgaagattccatgctgaaagcagagaacgtaccgggaccgggtaaacgtaccgaaatggggtgggaaatctcgcccgagtcactgtacgacttactgaaacgcttagaccgtgagtatacgaaactgccgatgtatatcaccgaaaatggagctgcgtttaaagatgaagtaacggaagatggtcgtgttcacgacgatgaacgcatcgaatacatcaaagagcacctgaaagctgccgctaaatttatcggggaaggcggtaatctgaaaggatactttgtgtggtcattaatggacaacttcgaatgggcgcatggctactccaaacgtttcggcattgtgtatgtggactatacgacccagaaacgcattctgaaggatagcgccttgtggtacaaagaggtgattcgtgatgatgggattgaagat

SEQ ID NO: 44 - protein, 447 aa, Thermoanaerobacter brockii
MAKFPRDFVWGTATSSYQIEGAVNEDGRTPSIWDTFSKTEGKTYKGHTGDVACDHYHRYKEDVEILKEIGVKAYRFSIAWPRIFPEEGKYNPKGMDFYKKLIDELQKRDIVPAATIYHWDLPQWAYDKGGGWLNRESIKWYVEYATKLFEELGDAIPLWITHNEPWCSSILSYGIGEHAPGHKNYREALIAAHHILLSHGEAVKAFREMNIKGSKIGITLNLTPAYPASEKEEDKLAAQYADGFANRWFLDPIFKGNYPEDMMELYSKIIGEFDFIKEGDLETISVPIDFLGVNYYTRSIVKYDEDSMLKAENVPGPGKRTEMGWEISPESLYDLLKRLDREYTKLPMYITENGAAFKDEVTEDGRVHDDERIEYIKEHLKAAAKFIGEGGNLKGYFVWSLMDNFEWAHGYSKRFGIVYVDYTTQKRILKDSALWYKEVILDDGIED

SEQ ID NO: 45 - DNA, 33 bp, Artificial Sequence
  Mutagenesis Primer
agcgcgatattaaacccgcagcgaccatttatc

SEQ ID NO: 46 - DNA, 33 bp, Artificial Sequence
  Mutagenesis Primer
gataaatggtcgctgcgggtttaatatcgcgct

SEQ ID NO: 47 - DNA, 33 bp, Artificial Sequence
  Mutragenesis Primer
cgattgacttcttaggcatcaattactacactc

SEQ ID NO: 48 - DNA, 33 bp, Artificial Sequence
  Mutagenesis Primer
gagtgtagtaattgatgcctaagaagtcaatcg

SEQ ID NO: 49 - DNA, 32 bp, Artificial Sequence
  Mutagenesis Primer
attgtgtatgtggactatgagacccagaaacg

SEQ ID NO: 50 - DNA, 32 bp, Artificial Sequence
  Mutegenesis Primer
cgtttctgggtctcatagtccacatacacaat

SEQ ID NO: 51 - DNA, 33 bp, Artificial Sequence
  Mutagenesis Primer
acaaagaggtgattcgcgatgatgggattgaag

SEQ ID NO: 52 - DNA, 33 bp, Artificial Sequence
  Mutagenesis Primer
cttcaatcccatcatcgcgaatcacctctttgt